European Patent Specification EP 3 431 999 B1, published July 26, 2023. Title: Method for Detecting Aggregate Form of Aggregate-Forming Polypeptides. Applicant: PeopleBio, Inc. The sequence listing filed with the application follows.

SEQUENCE LISTING (1 sequence)

SEQ ID NO: 1 - protein, 40 aa, Human amyloid beta
DAEFRHDSGYEVHHQKLVFFAEDVGCNKGAIIGLMVGGVV